European Patent Application EP 4 678 659 A1, published January 14, 2026. Title: MONOCLONAL ANTIBODY PREPARATION TARGETING TSLP. Applicant: 四川科伦博泰生物医药股份有限公司. Application CN. The sequence listing filed with the application follows.

SEQUENCE LISTING (17 sequences)

SEQ ID NO: 1 - protein, 8 aa, synthetic construct
  source 1..8: note = IMGT 43B1-H2L2 CDR-H1
GFTFRSYD

SEQ ID NO: 2 - protein, 8 aa, synthetic construct
  source 1..8: note = IMGT 43B1-H2L2 CDR-H2
IWYDGSNE

SEQ ID NO: 3 - protein, 16 aa, synthetic construct
  source 1..16: note = IMGT 43B1-H2L2 CDR-H3
ARSPLWYGEPDDAFDI

SEQ ID NO: 4 - protein, 6 aa, synthetic construct
  source 1..6: note = IMGT 43B1-H2L2 CDR-L1
QSVSSN

SEQ ID NO: 5 - skipped

SEQ ID NO: 6 - protein, 9 aa, synthetic construct
  source 1..9: note = IMGT/AbM 43B1-H2L2 CDR-L3
QHYNNWPLT

SEQ ID NO: 7 - protein, 10 aa, synthetic construct
  source 1..10: note = AbM 43B1-H2L2 CDR-H1
GFTFRSYDMH

SEQ ID NO: 8 - protein, 10 aa, synthetic construct
  source 1..10: note = AbM 43B1-H2L2 CDR-H2
VIWYDGSNEN

SEQ ID NO: 9 - protein, 14 aa, synthetic construct
  source 1..14: note = AbM 43B1-H2L2 CDR-H3
SPLWYGEPDDAFDI

SEQ ID NO: 10 - protein, 11 aa, synthetic construct
  source 1..11: note = AbM 43B1-H2L2 CDR-L1
RASQSVSSNLA

SEQ ID NO: 11 - protein, 7 aa, synthetic construct
  source 1..7: note = AbM 43B1-H2L2 CDR-L2
GASTRAT

SEQ ID NO: 12 - protein, 123 aa, synthetic construct
  source 1..123: note = VH of 43B1-H2L2
QMQLVESGGGAVQPGGSLRLSCAASGFTFRSYDMHWVRQAPGKGLEWVAVIWYDGSNENYADSVKGRFTTSRDNSKNTLFLQMNSLRAEDTAVYYCARSPLWYGEPDDAFDIWGQGTLVTVSS

SEQ ID NO: 13 - protein, 107 aa, synthetic construct
  source 1..107: note = VL of 43B1-H2L2
EIVMTQSPATLSVSPGERATLSCRASQSVSSNLAWYQQKPGQAPRLLISGASTRATGIPARFSGSGSGTDFTLTISSLQSEDFAVYYCQHYNNWPLTFGGGTKVEIK

SEQ ID NO: 14 - protein, 330 aa, synthetic construct
  source 1..330: note = modified human IgG1 heavy chain constant
ASTKGPSVFPLAPSSKSTSGGTAALGCLVKDYFPEPVTVSWNSGALTSGVHTFPAVLQSSGLYSLSSVVTVPSSSLGTQTYICNVNHKPSNTKVDKKVEPKSCDKTHTCPPCPAPEAAGAPSVFLFPPKPKDTLMISRTPEVTCVVVDVSHEDPEVKFNWYVDGVEVHNAKTKPREEQYNSTYRVVSVLTVLHQDWLNGKEYKCKVSNKALPAPIEKTISKAKGQPREPQVYTLPPSRDELTKNQVSLTCLVKGFYPSDIAVEWESNGQPENNYKTTPPVLDSDGSFFLYSKLTVDKSRWQQGNVFSCSVMHEALHAHYTQKSLSLSPGK

SEQ ID NO: 15 - protein, 107 aa, synthetic construct [sequence omitted]

SEQ ID NO: 16 - protein, 453 aa, synthetic construct
  source 1..453: note = heavy chain of 43B1-H2L2
QMQLVESGGGAVQPGGSLRLSCAASGFTFRSYDMHWVRQAPGKGLEWVAVIWYDGSNENYADSVKGRFTTSRDNSKNTLFLQMNSLRAEDTAVYYCARSPLWYGEPDDAFDIWGQGTLVTVSSASTKGPSVFPLAPSSKSTSGGTAALGCLVKDYFPEPVTVSWNSGALTSGVHTFPAVLQSSGLYSLSSVVTVPSSSLGTQTYICNVNHKPSNTKVDKKVEPKSCDKTHTCPPCPAPEAAGAPSVFLFPPKPKDTLMISRTPEVTCVVVDVSHEDPEVKFNWYVDGVEVHNAKTKPREEQYNSTYRVVSVLTVLHQDWLNGKEYKCKVSNKALPAPIEKTISKAKGQPREPQVYTLPPSRDELTKNQVSLTCLVKGFYPSDIAVEWESNGQPENNYKTTPPVLDSDGSFFLYSKLTVDKSRWQQGNVFSCSVMHEALHAHYTQKSLSLSPGK

SEQ ID NO: 17 - protein, 214 aa, synthetic construct
  source 1..214: note = light chain of 43B1-H2L2
EIVMTQSPATLSVSPGERATLSCRASQSVSSNLAWYQQKPGQAPRLLISGASTRATGIPARFSGSGSGTDFTLTISSLQSEDFAVYYCQHYNNWPLTFGGGTKVEIKRTVAAPSVFIFPPSDEQLKSGTASVVCLLNNFYPREAKVQWKVDNALQSGNSQESVTEQDSKDSTYSLSSTLTLSKADYEKHKVYACEVTHQGLSSPVTKSFNRGEC